European Patent Application EP 4 537 838 A1, published April 16, 2025. Title: Novel fragmented cysteinyl-tRNA synthetase peptide with immune-enhancing activity and use thereof. Applicant: Medicinal Bioconvergence Research Center. Application KR. The sequence listing filed with the application follows.

SEQUENCE LISTING (10 sequences)

SEQ ID NO: 1 - protein, 748 aa, synthetic construct
  REGION 1..748: note = cysteinyl-tRNA synthetase full length
MADSSGQQGKGRRVQPQWSPPAGTQPCRLHLYNSLTRNKEVFIPQDGKKVTWYCCGPTVYDASHMGHARSYISFDILRRVLKDYFKFDVFYCMNITDIDDKIIKRARQNHLFEQYREKRPEAAQLLEDVQAALKPFSVKLNETTDPDKKQMLERIQHAVQLATEPLEKAVQSRLTGEEVNSCVEVLLEEAKDLLSDWLDSTLGCDVTDNSIFSKLPKFWEGDFHRDMEALNVLPPDVLTRVSEYVPEIVNFVQKIVDNGYGYVSNGSVYFDTAKFASSEKHSYGKLVPEAVGDQKALQEGEGDLSISADRLSEKRSPNDFALWKASKPGEPSWPCPWGKGRPGWHIECSAMAGTLLGASMDIHGGGFDLRFPHHDNELAQSEAYFENDCWVRYFLHTGHLTIAGCKMSKSLKNFITIKDALKKHSARQLRLAFLMHSWKDTLDYSSNTMESALQYEKFLNEFFLNVKDILRAPVDITGQFEKWGEEEAELNKNFYDKKTAIHKALCDNVDTRTVMEEMRALVSQCNLYMAARKAVRKRPNQALLENIALYLTHMLKIFGAVEEDSSLGFPVGGPGTSLSLEATVMPYLQVLSEFREGVRKIAREQKVPEILQLSDALRDNILPELGVRFEDHEGLPTVVKLVDRNTLLKEREEKRRVEEEKRKKKEEAARRKQEQEAAKLAKMKIPPSEMFLSETDKYSKFDENGLPTHDMEGKELSKGQAKKLKKLFEAQEKLYKEYLQMAQNGSFQ

SEQ ID NO: 2 - protein, 61 aa, synthetic construct
  REGION 1..61: note = CRS 140-200
LNETTDPDKKQMLERIQHAVQLATEPLEKAVQSRLTGEEVNSCVEVLLEEAKDLLSDWLDS

SEQ ID NO: 3 - protein, 61 aa, synthetic construct
  REGION 1..61: note = CRS 140-200, C182S
LNETTDPDKKQMLERIQHAVQLATEPLEKAVQSRLTGEEVNSSVEVLLEEAKDLLSDWLDS

SEQ ID NO: 4 - protein, 123 aa, synthetic construct
  REGION 1..123: note = CRS 106-228
ARQNHLFEQYREKRPEAAQLLEDVQAALKPFSVKLNETTDPDKKQMLERIQHAVQLATEPLEKAVQSRLTGEEVNSCVEVLLEEAKDLLSDWLDSTLGCDVTDNSIFSKLPKFWEGDFHRDME

SEQ ID NO: 5 - protein, 100 aa, synthetic construct
  REGION 1..100: note = CRS 101-200
KIIKRARQNHLFEQYREKRPEAAQLLEDVQAALKPFSVKLNETTDPDKKQMLERIQHAVQLATEPLEKAVQSRLTGEEVNSCVEVLLEEAKDLLSDWLDS

SEQ ID NO: 6 - protein, 82 aa, synthetic construct
  REGION 1..82: note = CRS 119-200
RPEAAQLLEDVQAALKPFSVKLNETTDPDKKQMLERIQHAVQLATEPLEKAVQSRLTGEEVNSCVEVLLEEAKDLLSDWLDS

SEQ ID NO: 7 - protein, 102 aa, synthetic construct
  REGION 1..102: note = CRS 99-200
DDKIIKRARQNHLFEQYREKRPEAAQLLEDVQAALKPFSVKLNETTDPDKKQMLERIQHAVQLATEPLEKAVQSRLTGEEVNSCVEVLLEEAKDLLSDWLDS

SEQ ID NO: 8 - protein, 102 aa, synthetic construct
  REGION 1..102: note = CRS 99-200, C182S
DDKIIKRARQNHLFEQYREKRPEAAQLLEDVQAALKPFSVKLNETTDPDKKQMLERIQHAVQLATEPLEKAVQSRLTGEEVNSSVEVLLEEAKDLLSDWLDS

SEQ ID NO: 9 - DNA, 183 bp, synthetic construct
  misc_feature 1..183: note = CRS 140-200 polynucleotide
  source 1..183: mol_type = other DNA
ttaaatgagaccacggatcccgataaaaagcagatgctcgaacggattcagcacgcagtgcagcttgccacagagccacttgagaaagctgtgcagtccagactcacgggagaggaagtcaacagctgtgtggaggtgttgctggaagaagccaaggatttgctctctgactggctggattct

SEQ ID NO: 10 - DNA, 183 bp, synthetic construct
  misc_feature 1..183: note = CRS 140-200, C182S polynucleotide
  source 1..183: mol_type = other DNA
ttaaatgagaccacggatcccgataaaaagcagatgctcgaacggattcagcacgcagtgcagcttgccacagagccacttgagaaagctgtgcagtccagactcacgggagaggaagtcaacagcagtgtggaggtgttgctggaagaagccaaggatttgctctctgactggctggattct